European Patent Application EP 4 588 939 A1, published July 23, 2025. Title: INTERLEUKIN-13 RECEPTOR SUBUNIT ALPHA-2 (IL13Rα2) TARGETING MOIETIES FOR THE TREATMENT AND PREVENTION OF IL13Rα2-POSITIVE CANCER. Applicant: Universitat de Barcelona. The sequence listing filed with the application follows.

SEQUENCE LISTING (69 sequences)

SEQ ID NO: 1 - protein, 11 aa, synthetic construct
KASQDIKSYLS

SEQ ID NO: 2 - protein, 7 aa, synthetic construct
RANRLVD

SEQ ID NO: 3 - protein, 9 aa, synthetic construct
LQYDEFPLT

SEQ ID NO: 4 - protein, 5 aa, synthetic construct
EYTMH

SEQ ID NO: 5 - protein, 17 aa, synthetic construct
IINPNNGGTNYNQKFKG

SEQ ID NO: 6 - protein, 9 aa, synthetic construct
PSATHYFDY

SEQ ID NO: 7 - protein, 107 aa, synthetic construct
DIKMTQSPSSMYASLGERVTITCKASQDIKSYLSWFQQKPGKSPKTLIYRANRLVDGVPSRFSGSGSGQDYSLTISSLEYEDMGIYYCLQYDEFPLTFGAGTKLELK

SEQ ID NO: 8 - protein, 118 aa, synthetic construct
EVQLQQSGPELVKPGASVKISCKTSGYTFTEYTMHWVKQSHGKSLEWIGIINPNNGGTNYNQKFKGKATLTVDKSSSTAYMELRSLTSEDSAVYYCARPSATHYFDYWGQGTTLTVSS

SEQ ID NO: 9 - protein, 107 aa, synthetic construct
DIQMTQSPSSLYASVGDRVTITCKASQDIKSYLSWYQQKPGKAPKTLIYRANRLVDGVPSRFSGSGSGQDYTLTISSLQYEDMGIYYCLQYDEFPLTFGAGTKVEIK

SEQ ID NO: 10 - protein, 118 aa, synthetic construct
QVQLQQSGPEVVKPGASVKMSCKTSGYTFTEYTMHWVKQTHGRSLEWIGIINPNNGGTNYNQKFKGRATMTVDKSSSTAYMQLRSLTSDDTAVYYCARPSATHYFDYWGQGTTVTVSS

SEQ ID NO: 11 - DNA, 354 bp, synthetic construct
  source 1..354: mol_type = other DNA
gaagtccagcttcaacagtctgggcctgaattggtgaaacccggcgcgtccgttaaaatcagctgcaagacctctggatacacatttaccgagtatacaatgcattgggtaaagcagagccacggtaaaagtctggaatggatcggcattatcaatccaaataacgggggcactaattataaccagaaattcaaagggaaagctacactcaccgtggataagtcatcctcgacggcatatatggaactgcggtcccttacctcagaggattcagcagtctactattgtgcccgtccaagcgccacacactattttgactactggggacaaggaaccacactaactgtgtcttcg

SEQ ID NO: 12 - DNA, 321 bp, synthetic construct
  source 1..321: mol_type = other DNA
gacataaagatgacccagtcaccgtctagcatgtatgccagtctgggagagcgagtgactatcacatgcaaggccagccaggacataaagtcctacctcagttggttccaacagaagcctggcaagagtcccaaaactctgatttacagggctaacagactggttgacggggtgccctcccgcttctctggcagcggaagcggacaggattactccctgacgatctcctcactcgagtacgaggatatgggcatttactactgtttgcagtatgacgagtttcctttaactttcggagctggcaccaagctcgaactgaag

SEQ ID NO: 13 - protein, 268 aa, synthetic construct
MALPVTGLLLSLGLLLHAARPTGDIKMTQSPSSMYASLGERVTITCKASQDIKSYLSWFQQKPGKSPKTLIYRANRLVDGVPSRFSGSGSGQDYSLTISSLEYEDMGIYYCLQYDEFPLTFGAGTKLELKGGGGSGGGGSGGGGSGGGGSEVQLQQSGPELVKPGASVKISCKTSGYTFTEYTMHWVKQSHGKSLEWIGIINPNNGGTNYNQKFKGKATLTVDKSSSTAYMELRSLTSEDSAVYYCARPSATHYFDYWGQGTTLTVSS

SEQ ID NO: 14 - protein, 469 aa, synthetic construct
DIKMTQSPSSMYASLGERVTITCKASQDIKSYLSWFQQKPGKSPKTLIYRANRLVDGVPSRFSGSGSGQDYSLTISSLEYEDMGIYYCLQYDEFPLTFGAGTKLELKGGGGSGGGGSGGGGSGGGGSEVQLQQSGPELVKPGASVKISCKTSGYTFTEYTMHWVKQSHGKSLEWIGIINPNNGGTNYNQKFKGKATLTVDKSSSTAYMELRSLTSEDSAVYYCARPSATHYFDYWGQGTTLTVSSTTTPAPRPPTPAPTIASQPLSLRPEACRPAAGGAVHTRGLDFACDIYIWAPLAGTCGVLLLSLVITLYCKRGRKKLLYIFKQPFMRPVQTTQEEDGCSCRFPEEEEGGCELRVKFSRSADAPAYQQGQNQLYNELNLGRREEYDVLDKRRGRDPEMGGKPQRRKNPQEGLYNELQKDKMAEAYSEIGMKGERRRGKGHDGLYQGLSTATKDTYDALHMQALPPR

SEQ ID NO: 15 - protein, 268 aa, synthetic construct
MALPVTGLLLSLGLLLHAARPTGDIQMTQSPSSLYASVGDRVTITCKASQDIKSYLSWYQQKPGKAPKTLIYRANRLVDGVPSRFSGSGSGQDYTLTISSLQYEDMGIYYCLQYDEFPLTFGAGTKVEIKGGGGSGGGGSGGGGSGGGGSQVQLQQSGPEVVKPGASVKMSCKTSGYTFTEYTMHWVKQTHGRSLEWIGIINPNNGGTNYNQKFKGRATMTVDKSSSTAYMQLRSLTSDDTAVYYCARPSATHYFDYWGQGTTVTVSS

SEQ ID NO: 16 - protein, 469 aa, synthetic construct
DIQMTQSPSSLYASVGDRVTITCKASQDIKSYLSWYQQKPGKAPKTLIYRANRLVDGVPSRFSGSGSGQDYTLTISSLQYEDMGIYYCLQYDEFPLTFGAGTKVEIKGGGGSGGGGSGGGGSGGGGSQVQLQQSGPEVVKPGASVKMSCKTSGYTFTEYTMHWVKQTHGRSLEWIGIINPNNGGTNYNQKFKGRATMTVDKSSSTAYMQLRSLTSDDTAVYYCARPSATHYFDYWGQGTTVTVSSTTTPAPRPPTPAPTIASQPLSLRPEACRPAAGGAVHTRGLDFACDIYIWAPLAGTCGVLLLSLVITLYCKRGRKKLLYIFKQPFMRPVQTTQEEDGCSCRFPEEEEGGCELRVKFSRSADAPAYQQGQNQLYNELNLGRREEYDVLDKRRGRDPEMGGKPQRRKNPQEGLYNELQKDKMAEAYSEIGMKGERRRGKGHDGLYQGLSTATKDTYDALHMQALPPR

SEQ ID NO: 17 - protein, 12 aa, synthetic construct
TASSSVTSSYLH

SEQ ID NO: 18 - protein, 7 aa, synthetic construct
STSNLAS

SEQ ID NO: 19 - protein, 9 aa, synthetic construct
HQYHRSPLT

SEQ ID NO: 20 - protein, 5 aa, synthetic construct
KYGVH

SEQ ID NO: 21 - protein, 16 aa, synthetic construct
VIWSGGSTDYNAAFIS

SEQ ID NO: 22 - protein, 8 aa, synthetic construct
DFGDTMDY

SEQ ID NO: 23 - protein, 108 aa, synthetic construct
QIVLTQSPAIMSASLGERVTMTCTASSSVTSSYLHWYQQKPGSSPKLWIFSTSNLASGVPARFSGSGSGTSYSLTISSMEAEDAATYYCHQYHRSPLTFGAGTKLELK

SEQ ID NO: 24 - protein, 116 aa, synthetic construct
QVQLKQSGPGLVQPSQSLSITCTVSGFSITKYGVHWVRLSPGKGLEWLGVIWSGGSTDYNAAFISRLNISKDNSKSQVFFKMNSLQANDTAIYYCARDFGDTMDYWGQGTSVTVSS

SEQ ID NO: 25 - protein, 108 aa, synthetic construct
EIVLTQSPSILSASVGEDVTITCTASSSVTSSYLHWYQQKPGSAPKLWIYSTSNLASGVPSRFSGSGSGTSFTLTISSLQAEDAATYYCHQYHRSPLTFGAGTKLEIK

SEQ ID NO: 26 - protein, 116 aa, synthetic construct
QVQLQESGPGLVKPETSLSITCTVSGFSITKYGVHWVRLSPGKGLEWLGVIWSGGSTDYNAAFISRVNISKDNSKNQVFFKMNSLQANDTAVYYCARDFGDTMDYWGQGTTVTVSS

SEQ ID NO: 27 - protein, 324 aa, synthetic construct
CAAATCGTGCTGACGCAGAGTCCCGCCATCATGTCTGCAAGCCTGGGCGAGCGCGTGACCATGACTTGTACCGCCAGCAGCTCTGTTACATCTTCCTACCTCCACTGGTATCAGCAGAAGCCAGGCTCAAGTCCCAAGCTGTGGATTTTCAGTACTTCCAACTTAGCATCGGGTGTCCCTGCCCGATTCAGCGGGAGTGGGTCGGGAACTTCCTATTCATTGACCATTTCTTCCATGGAAGCGGAAGACGCCGCGACCTACTATTGCCATCAGTATCACAGAAGCCCGCTGACATTTGGCGCTGGAACAAAACTCGAGCTAAAG

SEQ ID NO: 28 - protein, 348 aa, synthetic construct
CAGGTGCAGCTGAAGCAGTCTGGACCTGGGTTGGTACAACCCTCCCAATCACTTAGCATCACATGCACGGTGTCAGGCTTTAGCATCACAAAGTACGGTGTGCATTGGGTTCGGCTGTCACCAGGAAAAGGGCTCGAGTGGCTTGGCGTGATTTGGAGTGGGGGAAGCACCGACTACAATGCAGCCTTCATAAGTAGGCTCAATATCTCAAAAGACAACTCTAAAAGTCAGGTATTCTTTAAGATGAATTCCCTGCAAGCCAACGATACCGCTATATACTACTGTGCTCGTGATTTTGGCGATACTATGGACTATTGGGGGCAGGGAACCAGCGTCACTGTCTCCTCC

SEQ ID NO: 29 - protein, 267 aa, synthetic construct
MALPVTGLLLSLGLLLHAARPTGQIVLTQSPAIMSASLGERVTMTCTASSSVTSSYLHWYQQKPGSSPKLWIFSTSNLASGVPARFSGSGSGTSYSLTISSMEAEDAATYYCHQYHRSPLTFGAGTKLELKGGGGSGGGGSGGGGSGGGGSQVQLKQSGPGLVQPSQSLSITCTVSGFSITKYGVHWVRLSPGKGLEWLGVIWSGGSTDYNAAFISRLNISKDNSKSQVFFKMNSLQANDTAIYYCARDFGDTMDYWGQGTSVTVSS

SEQ ID NO: 30 - protein, 468 aa, synthetic construct
QIVLTQSPAIMSASLGERVTMTCTASSSVTSSYLHWYQQKPGSSPKLWIFSTSNLASGVPARFSGSGSGTSYSLTISSMEAEDAATYYCHQYHRSPLTFGAGTKLELKGGGGSGGGGSGGGGSGGGGSQVQLKQSGPGLVQPSQSLSITCTVSGFSITKYGVHWVRLSPGKGLEWLGVIWSGGSTDYNAAFISRLNISKDNSKSQVFFKMNSLQANDTAIYYCARDFGDTMDYWGQGTSVTVSSTTTPAPRPPTPAPTIASQPLSLRPEACRPAAGGAVHTRGLDFACDIYIWAPLAGTCGVLLLSLVITLYCKRGRKKLLYIFKQPFMRPVQTTQEEDGCSCRFPEEEEGGCELRVKFSRSADAPAYQQGQNQLYNELNLGRREEYDVLDKRRGRDPEMGGKPQRRKNPQEGLYNELQKDKMAEAYSEIGMKGERRRGKGHDGLYQGLSTATKDTYDALHMQALPPR

SEQ ID NO: 31 - protein, 267 aa, synthetic construct
MALPVTGLLLSLGLLLHAARPTGEIVLTQSPSILSASVGEDVTITCTASSSVTSSYLHWYQQKPGSAPKLWIYSTSNLASGVPSRFSGSGSGTSFTLTISSLQAEDAATYYCHQYHRSPLTFGAGTKLEIKGGGGSGGGGSGGGGSGGGGSQVQLQESGPGLVKPETSLSITCTVSGFSITKYGVHWVRLSPGKGLEWLGVIWSGGSTDYNAAFISRVNISKDNSKNQVFFKMNSLQANDTAVYYCARDFGDTMDYWGQGTTVTVSS

SEQ ID NO: 32 - protein, 468 aa, synthetic construct
EIVLTQSPSILSASVGEDVTITCTASSSVTSSYLHWYQQKPGSAPKLWIYSTSNLASGVPSRFSGSGSGTSFTLTISSLQAEDAATYYCHQYHRSPLTFGAGTKLEIKGGGGSGGGGSGGGGSGGGGSQVQLQESGPGLVKPETSLSITCTVSGFSITKYGVHWVRLSPGKGLEWLGVIWSGGSTDYNAAFISRVNISKDNSKNQVFFKMNSLQANDTAVYYCARDFGDTMDYWGQGTTVTVSSTTTPAPRPPTPAPTIASQPLSLRPEACRPAAGGAVHTRGLDFACDIYIWAPLAGTCGVLLLSLVITLYCKRGRKKLLYIFKQPFMRPVQTTQEEDGCSCRFPEEEEGGCELRVKFSRSADAPAYQQGQNQLYNELNLGRREEYDVLDKRRGRDPEMGGKPQRRKNPQEGLYNELQKDKMAEAYSEIGMKGERRRGKGHDGLYQGLSTATKDTYDALHMQALPPR

SEQ ID NO: 33 - protein, 11 aa, synthetic construct
KASQDINSYLS

SEQ ID NO: 34 - protein, 7 aa, synthetic construct
RANRLVD

SEQ ID NO: 35 - protein, 9 aa, synthetic construct
LQYDEFPLT

SEQ ID NO: 36 - protein, 5 aa, synthetic construct
SFGMH

SEQ ID NO: 37 - protein, 17 aa, synthetic construct
YISSGSSTIYYADTVKG

SEQ ID NO: 38 - protein, 9 aa, synthetic construct
KYEGYAMDY

SEQ ID NO: 39 - protein, 107 aa, synthetic construct
DIKMTQSPSSMYASLGERVTITCKASQDINSYLSWFQQKPGKSPKTLIYRANRLVDGVPSRFSGSGSGQDYSLTISSLEYEDMGIYSCLQYDEFPLTFGAGTKLELK

SEQ ID NO: 40 - protein, 118 aa, synthetic construct
DVQLVESGGGLVQPGGSRKLSCAASGFTFSSFGMHWVRQAPEKGLEWVAYISSGSSTIYYADTVKGRFIISRDNPKNTLFLQMTSLRSEDTAMYYCARKYEGYAMDYWGQGTSVTVSS

SEQ ID NO: 41 - protein, 107 aa, synthetic construct
DIQMTQSPSSLYASVGDRVTITCKASQDINSYLSWYQQKPGKAPKTLIYRANRLVDGVPSRFSGSGSGQDYTLTISSLQYEDMGIYSCLQYDEFPLTFGAGTKVEIK

SEQ ID NO: 42 - protein, 118 aa, synthetic construct
EVQLVESGGGLVQPGGSLKLSCAASGFTFSSFGMHWVRQAPEKGLEWVAYISSGSSTIYYADTVKGRFIISRDNPKNTLFLQMTSLRSEDTAMYYCARKYEGYAMDYWGQGTLVTVSS

SEQ ID NO: 43 - protein, 354 aa, synthetic construct
GACGTGCAGCTGGTGGAAAGTGGAGGCGGTCTCGTCCAGCCAGGTGGTAGCAGAAAGTTGAGCTGTGCCGCCAGTGGTTTTACATTCAGCTCCTTCGGAATGCACTGGGTTCGTCAGGCACCCGAAAAGGGCCTGGAGTGGGTGGCCTATATATCCAGCGGCAGTTCTACAATCTATTATGCCGACACAGTCAAAGGTAGGTTCATTATCTCCCGCGATAATCCCAAGAACACCCTGTTCTTACAGATGACCTCACTGCGGTCTGAGGATACAGCTATGTACTACTGCGCTAGAAAATATGAGGGCTATGCTATGGACTACTGGGGACAGGGGACTTCCGTCACCGTGTCGTCG

SEQ ID NO: 44 - DNA, 321 bp, synthetic construct
  source 1..321: mol_type = other DNA
gatatcaagatgacccaatcaccttcttcaatgtatgcaagtcttggcgaaagggtaactattacttgcaaggcctcccaagacatcaactcttacctctcctggtttcagcagaaacctggcaagagtcccaaaacgctgatctaccgggcaaatcgcttggttgacggtgtgccgagccgattttcagggagcgggtctggacaggactacagccttacgatttcttctctggagtacgaggatatgggaatatactcctgtctccaatatgatgagtttccactcaccttcggggcggggactaagctggaactaaaa

SEQ ID NO: 45 - protein, 268 aa, synthetic construct
MALPVTGLLLSLGLLLHAARPTGDIKMTQSPSSMYASLGERVTITCKASQDINSYLSWFQQKPGKSPKTLIYRANRLVDGVPSRFSGSGSGQDYSLTISSLEYEDMGIYSCLQYDEFPLTFGAGTKLELKGGGGSGGGGSGGGGSGGGGSDVQLVESGGGLVQPGGSRKLSCAASGFTFSSFGMHWVRQAPEKGLEWVAYISSGSSTIYYADTVKGRFIISRDNPKNTLFLQMTSLRSEDTAMYYCARKYEGYAMDYWGQGTSVTVSS

SEQ ID NO: 46 - protein, 469 aa, synthetic construct
DIKMTQSPSSMYASLGERVTITCKASQDINSYLSWFQQKPGKSPKTLIYRANRLVDGVPSRFSGSGSGQDYSLTISSLEYEDMGIYSCLQYDEFPLTFGAGTKLELKGGGGSGGGGSGGGGSGGGGSDVQLVESGGGLVQPGGSRKLSCAASGFTFSSFGMHWVRQAPEKGLEWVAYISSGSSTIYYADTVKGRFIISRDNPKNTLFLQMTSLRSEDTAMYYCARKYEGYAMDYWGQGTSVTVSSTTTPAPRPPTPAPTIASQPLSLRPEACRPAAGGAVHTRGLDFACDIYIWAPLAGTCGVLLLSLVITLYCKRGRKKLLYIFKQPFMRPVQTTQEEDGCSCRFPEEEEGGCELRVKFSRSADAPAYQQGQNQLYNELNLGRREEYDVLDKRRGRDPEMGGKPQRRKNPQEGLYNELQKDKMAEAYSEIGMKGERRRGKGHDGLYQGLSTATKDTYDALHMQALPPR

SEQ ID NO: 47 - protein, 268 aa, synthetic construct
MALPVTGLLLSLGLLLHAARPTGDIQMTQSPSSLYASVGDRVTITCKASQDINSYLSWYQQKPGKAPKTLIYRANRLVDGVPSRFSGSGSGQDYTLTISSLQYEDMGIYSCLQYDEFPLTFGAGTKVEIKGGGGSGGGGSGGGGSGGGGSEVQLVESGGGLVQPGGSLKLSCAASGFTFSSFGMHWVRQAPEKGLEWVAYISSGSSTIYYADTVKGRFIISRDNPKNTLFLQMTSLRSEDTAMYYCARKYEGYAMDYWGQGTLVTVSS

SEQ ID NO: 48 - protein, 469 aa, synthetic construct
DIQMTQSPSSLYASVGDRVTITCKASQDINSYLSWYQQKPGKAPKTLIYRANRLVDGVPSRFSGSGSGQDYTLTISSLQYEDMGIYSCLQYDEFPLTFGAGTKVEIKGGGGSGGGGSGGGGSGGGGSEVQLVESGGGLVQPGGSLKLSCAASGFTFSSFGMHWVRQAPEKGLEWVAYISSGSSTIYYADTVKGRFIISRDNPKNTLFLQMTSLRSEDTAMYYCARKYEGYAMDYWGQGTLVTVSSTTTPAPRPPTPAPTIASQPLSLRPEACRPAAGGAVHTRGLDFACDIYIWAPLAGTCGVLLLSLVITLYCKRGRKKLLYIFKQPFMRPVQTTQEEDGCSCRFPEEEEGGCELRVKFSRSADAPAYQQGQNQLYNELNLGRREEYDVLDKRRGRDPEMGGKPQRRKNPQEGLYNELQKDKMAEAYSEIGMKGERRRGKGHDGLYQGLSTATKDTYDALHMQALPPR

SEQ ID NO: 49 - protein, 12 aa, synthetic construct
TASSSVSSSYLH

SEQ ID NO: 50 - protein, 7 aa, synthetic construct
STSNLAS

SEQ ID NO: 51 - protein, 9 aa, synthetic construct
HQYHRSPLT

SEQ ID NO: 52 - protein, 5 aa, synthetic construct
SYGVH

SEQ ID NO: 53 - protein, 16 aa, synthetic construct
VIWSGGSTDYNAAFIS

SEQ ID NO: 54 - protein, 8 aa, synthetic construct
DRYDAFDY

SEQ ID NO: 55 - protein, 108 aa, synthetic construct
QIVLTQSPAIMSASLGERVTMTCTASSSVSSSYLHWYQQKPGSSPKLWIYSTSNLASGVPARFSGSGSGTSYSLTISSMEAEDAATYYCHQYHRSPLTFGAGTKLELK

SEQ ID NO: 56 - protein, 116 aa, synthetic construct
QVQLKQSGPGLVQPSQSLSITCTVSGFSLTSYGVHWVRQSPGKGLEWLGVIWSGGSTDYNAAFISRLSISKDNSKSQVFFKMNSLQANDTAIYYCARDRYDAFDYWGQGTTLTVSS

SEQ ID NO: 57 - protein, 108 aa, synthetic construct
EIVLTQSPSILSASVGEDVTITCTASSSVSSSYLHWYQQKPGSAPKLWIYSTSNLASGVPSRFSGSGSGTSFTLTISSLQAEDAATYYCHQYHRSPLTFGAGTKLEIK

SEQ ID NO: 58 - protein, 116 aa, synthetic construct
QVQLQESGPGLVRPSQSLSLTCTVSGFSLTSYGVHWVRQSPGRGLEWLGVIWSGGSTDYNAAFISRVTMSKDNSKNQVFFRMNSLQANDTAVYYCARDRYDAFDYWGQGTTVTVSS

SEQ ID NO: 59 - DNA, 348 bp, synthetic construct
  source 1..348: mol_type = other DNA
caggttcaacttaaacagtctggacccggactggttcagccaagtcagagcctatccatcacctgtacagtaagcggtttctccctcacctcctatggggtgcattgggtgcgacagtctcctgggaaggggctggaatggttgggcgtcatctggagcgggggcagcaccgattacaatgctgccttcatttcaaggctcagcatcagtaaagacaatagcaagtcccaggtcttcttcaaaatgaacagtctgcaggcgaacgacacagccatatactactgtgcccgtgaccggtatgatgcgtttgattattgggggcaaggaactacgctgaccgtgagcagt

SEQ ID NO: 60 - DNA, 324 bp, synthetic construct
  source 1..324: mol_type = other DNA
caaatagtgctcacacaatcacccgcaattatgtccgcatctctgggagaaagagtgacaatgacgtgcaccgcatcatcttctgtctccagttcctacctccactggtatcagcagaagcccggctcaagcccaaagttatggatttactctactagcaacttagcctccggcgtgcctgctcgcttttccggttcgggctctggcacctcatattcgttgactatctcttcaatggaggctgaggacgctgccacttattactgccatcagtaccacaggtcaccgctgacttttggcgccgggacaaaactggagcttaag

SEQ ID NO: 61 - protein, 267 aa, synthetic construct
MALPVTGLLLSLGLLLHAARPTGQIVLTQSPAIMSASLGERVTMTCTASSSVSSSYLHWYQQKPGSSPKLWIYSTSNLASGVPARFSGSGSGTSYSLTISSMEAEDAATYYCHQYHRSPLTFGAGTKLELKGGGGSGGGGSGGGGSGGGGSQVQLKQSGPGLVQPSQSLSITCTVSGFSLTSYGVHWVRQSPGKGLEWLGVIWSGGSTDYNAAFISRLSISKDNSKSQVFFKMNSLQANDTAIYYCARDRYDAFDYWGQGTTLTVSS

SEQ ID NO: 62 - protein, 468 aa, synthetic construct
QIVLTQSPAIMSASLGERVTMTCTASSSVSSSYLHWYQQKPGSSPKLWIYSTSNLASGVPARFSGSGSGTSYSLTISSMEAEDAATYYCHQYHRSPLTFGAGTKLELKGGGGSGGGGSGGGGSGGGGSQVQLKQSGPGLVQPSQSLSITCTVSGFSLTSYGVHWVRQSPGKGLEWLGVIWSGGSTDYNAAFISRLSISKDNSKSQVFFKMNSLQANDTAIYYCARDRYDAFDYWGQGTTLTVSSTTTPAPRPPTPAPTIASQPLSLRPEACRPAAGGAVHTRGLDFACDIYIWAPLAGTCGVLLLSLVITLYCKRGRKKLLYIFKQPFMRPVQTTQEEDGCSCRFPEEEEGGCELRVKFSRSADAPAYQQGQNQLYNELNLGRREEYDVLDKRRGRDPEMGGKPQRRKNPQEGLYNELQKDKMAEAYSEIGMKGERRRGKGHDGLYQGLSTATKDTYDALHMQALPPR

SEQ ID NO: 63 - protein, 267 aa, synthetic construct
MALPVTGLLLSLGLLLHAARPTGEIVLTQSPSILSASVGEDVTITCTASSSVSSSYLHWYQQKPGSAPKLWIYSTSNLASGVPSRFSGSGSGTSFTLTISSLQAEDAATYYCHQYHRSPLTFGAGTKLEIKGGGGSGGGGSGGGGSGGGGSQVQLQESGPGLVRPSQSLSLTCTVSGFSLTSYGVHWVRQSPGRGLEWLGVIWSGGSTDYNAAFISRVTMSKDNSKNQVFFRMNSLQANDTAVYYCARDRYDAFDYWGQGTTVTVSS

SEQ ID NO: 64 - protein, 468 aa, synthetic construct
EIVLTQSPSILSASVGEDVTITCTASSSVSSSYLHWYQQKPGSAPKLWIYSTSNLASGVPSRFSGSGSGTSFTLTISSLQAEDAATYYCHQYHRSPLTFGAGTKLEIKGGGGSGGGGSGGGGSGGGGSQVQLQESGPGLVRPSQSLSLTCTVSGFSLTSYGVHWVRQSPGRGLEWLGVIWSGGSTDYNAAFISRVTMSKDNSKNQVFFRMNSLQANDTAVYYCARDRYDAFDYWGQGTTVTVSSTTTPAPRPPTPAPTIASQPLSLRPEACRPAAGGAVHTRGLDFACDIYIWAPLAGTCGVLLLSLVITLYCKRGRKKLLYIFKQPFMRPVQTTQEEDGCSCRFPEEEEGGCELRVKFSRSADAPAYQQGQNQLYNELNLGRREEYDVLDKRRGRDPEMGGKPQRRKNPQEGLYNELQKDKMAEAYSEIGMKGERRRGKGHDGLYQGLSTATKDTYDALHMQALPPR

SEQ ID NO: 65 - protein, 20 aa, synthetic construct
GGGGSGGGGSGGGGSGGGGS

SEQ ID NO: 66 - protein, 23 aa, synthetic construct
MALPVTGLLLSLGLLLHAARPTG

SEQ ID NO: 67 - protein, 69 aa, synthetic construct
TTTPAPRPPTPAPTIASQPLSLRPEACRPAAGGAVHTRGLDFACDIYIWAPLAGTCGVLLLSLVITLYC

SEQ ID NO: 68 - protein, 113 aa, synthetic construct
RVKFSRSADAPAYQQGQNQLYNELNLGRREEYDVLDKRRGRDPEMGGKPQRRKNPQEGLYNELQKDKMAEAYSEIGMKGERRRGKGHDGLYQGLSTATKDTYDALHMQALPPR

SEQ ID NO: 69 - protein, 42 aa, synthetic construct
KRGRKKLLYIFKQPFMRPVQTTQEEDGCSCRFPEEEEGGCEL